European Patent Specification EP 3 897 845 B1, published January 14, 2026. Title: BIFUNCTIONAL MOLECULE DIRECTED AGAINST HUMAN PD-1. Applicant: OSE IMMUNOTHERAPEUTICS. The sequence listing filed with the application follows.

SEQUENCE LISTING (62 sequences)

SEQ ID NO: 1 - protein, 5 aa, artificial
  HC CDR1
HYAMN

SEQ ID NO: 2 - protein, 17 aa, artificial
  HC CDR2
WINTNTGEPTYAQGFTG

SEQ ID NO: 3 - protein, 8 aa, artificial
  HC CDR3
  MISC_FEATURE (7)..(7): X is X1 (D or E)
  MISC_FEATURE (8)..(8): X is X2 and is T, H, A, Y, N, E or S
EREPGMXX

SEQ ID NO: 4 - protein, 8 aa, artificial
  HC CDR3
EREPGMDS

SEQ ID NO: 5 - protein, 8 aa, artificial
  HC CDR3
EREPGMDT

SEQ ID NO: 6 - protein, 8 aa, artificial
  HC CDR3
EREPGMES

SEQ ID NO: 7 - protein, 8 aa, artificial
  HC CDR3
EREPGMDH

SEQ ID NO: 8 - protein, 8 aa, artificial
  HC CDR3
EREPGMDA

SEQ ID NO: 9 - protein, 8 aa, artificial
  HC CDR3
EREPGMDY

SEQ ID NO: 10 - protein, 8 aa, artificial
  HC CDR3
EREPGMDN

SEQ ID NO: 11 - protein, 8 aa, artificial
  HC CDR3
EREPGMDE

SEQ ID NO: 12 - protein, 16 aa, artificial
  LC CDR1
  MISC_FEATURE (11)..(11): X is G or T
RSSQSLVHANXNTYLE

SEQ ID NO: 13 - protein, 16 aa, artificial
  LC CDR1
RSSQSLVHANGNTYLE

SEQ ID NO: 14 - protein, 16 aa, artificial
  LC CDR1
RSSQSLVHANTNTYLE

SEQ ID NO: 15 - protein, 7 aa, artificial
  LC CDR2
KVSNRFS

SEQ ID NO: 16 - protein, 9 aa, artificial
  LC CDR3
FQGTHVPNT

SEQ ID NO: 17 - protein, 117 aa, artificial
  HC variable domain
  MISC_FEATURE (105)..(105): X is X1, D or E
  MISC_FEATURE (106)..(106): X is X2 and is T, H, A, Y, N, E or S
QIQLVQSGSELKKPGASVKVSCKASGYTFTHYAMNWVRQAPGQGLEWMGWINTNTGEPTYAQGFTGRFVFSLDTSVSTAYLQISSLKAEDTAVYYCAREREPGMXXWGQGTLVTVSS

SEQ ID NO: 18 - protein, 117 aa, artificial
  HC variable domain
QIQLVQSGSELKKPGASVKVSCKASGYTFTHYAMNWVRQAPGQGLEWMGWINTNTGEPTYAQGFTGRFVFSLDTSVSTAYLQISSLKAEDTAVYYCAREREPGMDSWGQGTLVTVSS

SEQ ID NO: 19 - protein, 117 aa, artificial
  HC variable domain
QIQLVQSGSELKKPGASVKVSCKASGYTFTHYAMNWVRQAPGQGLEWMGWINTNTGEPTYAQGFTGRFVFSLDTSVSTAYLQISSLKAEDTAVYYCAREREPGMDTWGQGTLVTVSS

SEQ ID NO: 20 - protein, 117 aa, artificial
  HC variable domain
QIQLVQSGSELKKPGASVKVSCKASGYTFTHYAMNWVRQAPGQGLEWMGWINTNTGEPTYAQGFTGRFVFSLDTSVSTAYLQISSLKAEDTAVYYCAREREPGMESWGQGTLVTVSS

SEQ ID NO: 21 - protein, 117 aa, artificial
  HC variable domain
QIQLVQSGSELKKPGASVKVSCKASGYTFTHYAMNWVRQAPGQGLEWMGWINTNTGEPTYAQGFTGRFVFSLDTSVSTAYLQISSLKAEDTAVYYCAREREPGMDHWGQGTLVTVSS

SEQ ID NO: 22 - protein, 117 aa, artificial
  HC variable domain
QIQLVQSGSELKKPGASVKVSCKASGYTFTHYAMNWVRQAPGQGLEWMGWINTNTGEPTYAQGFTGRFVFSLDTSVSTAYLQISSLKAEDTAVYYCAREREPGMDAWGQGTLVTVSS

SEQ ID NO: 23 - protein, 117 aa, artificial
  HC variable domain
QIQLVQSGSELKKPGASVKVSCKASGYTFTHYAMNWVRQAPGQGLEWMGWINTNTGEPTYAQGFTGRFVFSLDTSVSTAYLQISSLKAEDTAVYYCAREREPGMDYWGQGTLVTVSS

SEQ ID NO: 24 - protein, 117 aa, artificial
  HC variable domain
QIQLVQSGSELKKPGASVKVSCKASGYTFTHYAMNWVRQAPGQGLEWMGWINTNTGEPTYAQGFTGRFVFSLDTSVSTAYLQISSLKAEDTAVYYCAREREPGMDNWGQGTLVTVSS

SEQ ID NO: 25 - protein, 117 aa, artificial
  HC variable domain
QIQLVQSGSELKKPGASVKVSCKASGYTFTHYAMNWVRQAPGQGLEWMGWINTNTGEPTYAQGFTGRFVFSLDTSVSTAYLQISSLKAEDTAVYYCAREREPGMDEWGQGTLVTVSS

SEQ ID NO: 26 - protein, 112 aa, artificial
  LC variable domain
  MISC_FEATURE (34)..(34): X is G or T
DVVMTQSPLSLPVTLGQPASISCRSSQSLVHANXNTYLEWYQQRPGQSPRLLIYKVSNRFSGVPDRFSGSGSGTDFTLKISRVEAEDVGVYYCFQGTHVPNTFGQGTKLEIK

SEQ ID NO: 27 - protein, 112 aa, artificial
  LC variable domain
DVVMTQSPLSLPVTLGQPASISCRSSQSLVHANGNTYLEWYQQRPGQSPRLLIYKVSNRFSGVPDRFSGSGSGTDFTLKISRVEAEDVGVYYCFQGTHVPNTFGQGTKLEIK

SEQ ID NO: 28 - protein, 112 aa, artificial
  LC variable domain
DVVMTQSPLSLPVTLGQPASISCRSSQSLVHANTNTYLEWYQQRPGQSPRLLIYKVSNRFSGVPDRFSGSGSGTDFTLKISRVEAEDVGVYYCFQGTHVPNTFGQGTKLEIK

SEQ ID NO: 29 - protein, 444 aa, artificial
  HC
QIQLVQSGSELKKPGASVKVSCKASGYTFTHYAMNWVRQAPGQGLEWMGWINTNTGEPTYAQGFTGRFVFSLDTSVSTAYLQISSLKAEDTAVYYCAREREPGMDSWGQGTLVTVSSASTKGPSVFPLAPCSRSTSESTAALGCLVKDYFPEPVTVSWNSGALTSGVHTFPAVLQSSGLYSLSSVVTVPSSSLGTKTYTCNVDHKPSNTKVDKRVESKYGPPCPPCPAPEFLGGPSVFLFPPKPKDTLMISRTPEVTCVVVDVSQEDPEVQFNWYVDGVEVHNAKTKPREEQFNSTYRVVSVLTVLHQDWLNGKEYKCKVSNKGLPSSIEKTISKAKGQPREPQVYTLPPSQEEMTKNQVSLTCLVKGFYPSDIAVEWESNGQPENNYKTTPPVLDSDGSFFLYSRLTVDKSRWQEGNVFSCSVMHEALHNHYTQKSLSLSPGK

SEQ ID NO: 30 - protein, 444 aa, artificial
  HC
QIQLVQSGSELKKPGASVKVSCKASGYTFTHYAMNWVRQAPGQGLEWMGWINTNTGEPTYAQGFTGRFVFSLDTSVSTAYLQISSLKAEDTAVYYCAREREPGMDTWGQGTLVTVSSASTKGPSVFPLAPCSRSTSESTAALGCLVKDYFPEPVTVSWNSGALTSGVHTFPAVLQSSGLYSLSSVVTVPSSSLGTKTYTCNVDHKPSNTKVDKRVESKYGPPCPPCPAPEFLGGPSVFLFPPKPKDTLMISRTPEVTCVVVDVSQEDPEVQFNWYVDGVEVHNAKTKPREEQFNSTYRVVSVLTVLHQDWLNGKEYKCKVSNKGLPSSIEKTISKAKGQPREPQVYTLPPSQEEMTKNQVSLTCLVKGFYPSDIAVEWESNGQPENNYKTTPPVLDSDGSFFLYSRLTVDKSRWQEGNVFSCSVMHEALHNHYTQKSLSLSPGK

SEQ ID NO: 31 - protein, 444 aa, artificial
  HC
QIQLVQSGSELKKPGASVKVSCKASGYTFTHYAMNWVRQAPGQGLEWMGWINTNTGEPTYAQGFTGRFVFSLDTSVSTAYLQISSLKAEDTAVYYCAREREPGMESWGQGTLVTVSSASTKGPSVFPLAPCSRSTSESTAALGCLVKDYFPEPVTVSWNSGALTSGVHTFPAVLQSSGLYSLSSVVTVPSSSLGTKTYTCNVDHKPSNTKVDKRVESKYGPPCPPCPAPEFLGGPSVFLFPPKPKDTLMISRTPEVTCVVVDVSQEDPEVQFNWYVDGVEVHNAKTKPREEQFNSTYRVVSVLTVLHQDWLNGKEYKCKVSNKGLPSSIEKTISKAKGQPREPQVYTLPPSQEEMTKNQVSLTCLVKGFYPSDIAVEWESNGQPENNYKTTPPVLDSDGSFFLYSRLTVDKSRWQEGNVFSCSVMHEALHNHYTQKSLSLSPGK

SEQ ID NO: 32 - protein, 444 aa, artificial
  HC
QIQLVQSGSELKKPGASVKVSCKASGYTFTHYAMNWVRQAPGQGLEWMGWINTNTGEPTYAQGFTGRFVFSLDTSVSTAYLQISSLKAEDTAVYYCAREREPGMDHWGQGTLVTVSSASTKGPSVFPLAPCSRSTSESTAALGCLVKDYFPEPVTVSWNSGALTSGVHTFPAVLQSSGLYSLSSVVTVPSSSLGTKTYTCNVDHKPSNTKVDKRVESKYGPPCPPCPAPEFLGGPSVFLFPPKPKDTLMISRTPEVTCVVVDVSQEDPEVQFNWYVDGVEVHNAKTKPREEQFNSTYRVVSVLTVLHQDWLNGKEYKCKVSNKGLPSSIEKTISKAKGQPREPQVYTLPPSQEEMTKNQVSLTCLVKGFYPSDIAVEWESNGQPENNYKTTPPVLDSDGSFFLYSRLTVDKSRWQEGNVFSCSVMHEALHNHYTQKSLSLSPGK

SEQ ID NO: 33 - protein, 444 aa, artificial
  HC
QIQLVQSGSELKKPGASVKVSCKASGYTFTHYAMNWVRQAPGQGLEWMGWINTNTGEPTYAQGFTGRFVFSLDTSVSTAYLQISSLKAEDTAVYYCAREREPGMDAWGQGTLVTVSSASTKGPSVFPLAPCSRSTSESTAALGCLVKDYFPEPVTVSWNSGALTSGVHTFPAVLQSSGLYSLSSVVTVPSSSLGTKTYTCNVDHKPSNTKVDKRVESKYGPPCPPCPAPEFLGGPSVFLFPPKPKDTLMISRTPEVTCVVVDVSQEDPEVQFNWYVDGVEVHNAKTKPREEQFNSTYRVVSVLTVLHQDWLNGKEYKCKVSNKGLPSSIEKTISKAKGQPREPQVYTLPPSQEEMTKNQVSLTCLVKGFYPSDIAVEWESNGQPENNYKTTPPVLDSDGSFFLYSRLTVDKSRWQEGNVFSCSVMHEALHNHYTQKSLSLSPGK

SEQ ID NO: 34 - protein, 444 aa, artificial
  HC
QIQLVQSGSELKKPGASVKVSCKASGYTFTHYAMNWVRQAPGQGLEWMGWINTNTGEPTYAQGFTGRFVFSLDTSVSTAYLQISSLKAEDTAVYYCAREREPGMDYWGQGTLVTVSSASTKGPSVFPLAPCSRSTSESTAALGCLVKDYFPEPVTVSWNSGALTSGVHTFPAVLQSSGLYSLSSVVTVPSSSLGTKTYTCNVDHKPSNTKVDKRVESKYGPPCPPCPAPEFLGGPSVFLFPPKPKDTLMISRTPEVTCVVVDVSQEDPEVQFNWYVDGVEVHNAKTKPREEQFNSTYRVVSVLTVLHQDWLNGKEYKCKVSNKGLPSSIEKTISKAKGQPREPQVYTLPPSQEEMTKNQVSLTCLVKGFYPSDIAVEWESNGQPENNYKTTPPVLDSDGSFFLYSRLTVDKSRWQEGNVFSCSVMHEALHNHYTQKSLSLSPGK

SEQ ID NO: 35 - protein, 444 aa, artificial
  HC
QIQLVQSGSELKKPGASVKVSCKASGYTFTHYAMNWVRQAPGQGLEWMGWINTNTGEPTYAQGFTGRFVFSLDTSVSTAYLQISSLKAEDTAVYYCAREREPGMDNWGQGTLVTVSSASTKGPSVFPLAPCSRSTSESTAALGCLVKDYFPEPVTVSWNSGALTSGVHTFPAVLQSSGLYSLSSVVTVPSSSLGTKTYTCNVDHKPSNTKVDKRVESKYGPPCPPCPAPEFLGGPSVFLFPPKPKDTLMISRTPEVTCVVVDVSQEDPEVQFNWYVDGVEVHNAKTKPREEQFNSTYRVVSVLTVLHQDWLNGKEYKCKVSNKGLPSSIEKTISKAKGQPREPQVYTLPPSQEEMTKNQVSLTCLVKGFYPSDIAVEWESNGQPENNYKTTPPVLDSDGSFFLYSRLTVDKSRWQEGNVFSCSVMHEALHNHYTQKSLSLSPGK

SEQ ID NO: 36 - protein, 444 aa, artificial
  HC
QIQLVQSGSELKKPGASVKVSCKASGYTFTHYAMNWVRQAPGQGLEWMGWINTNTGEPTYAQGFTGRFVFSLDTSVSTAYLQISSLKAEDTAVYYCAREREPGMDEWGQGTLVTVSSASTKGPSVFPLAPCSRSTSESTAALGCLVKDYFPEPVTVSWNSGALTSGVHTFPAVLQSSGLYSLSSVVTVPSSSLGTKTYTCNVDHKPSNTKVDKRVESKYGPPCPPCPAPEFLGGPSVFLFPPKPKDTLMISRTPEVTCVVVDVSQEDPEVQFNWYVDGVEVHNAKTKPREEQFNSTYRVVSVLTVLHQDWLNGKEYKCKVSNKGLPSSIEKTISKAKGQPREPQVYTLPPSQEEMTKNQVSLTCLVKGFYPSDIAVEWESNGQPENNYKTTPPVLDSDGSFFLYSRLTVDKSRWQEGNVFSCSVMHEALHNHYTQKSLSLSPGK

SEQ ID NO: 37 - protein, 219 aa, artificial
  LC
DVVMTQSPLSLPVTLGQPASISCRSSQSLVHANGNTYLEWYQQRPGQSPRLLIYKVSNRFSGVPDRFSGSGSGTDFTLKISRVEAEDVGVYYCFQGTHVPNTFGQGTKLEIKRTVAAPSVFIFPPSDEQLKSGTASVVCLLNNFYPREAKVQWKVDNALQSGNSQESVTEQDSKDSTYSLSSTLTLSKADYEKHKVYACEVTHQGLSSPVTKSFNRGEC

SEQ ID NO: 38 - protein, 219 aa, artificial
  LC
DVVMTQSPLSLPVTLGQPASISCRSSQSLVHANTNTYLEWYQQRPGQSPRLLIYKVSNRFSGVPDRFSGSGSGTDFTLKISRVEAEDVGVYYCFQGTHVPNTFGQGTKLEIKRTVAAPSVFIFPPSDEQLKSGTASVVCLLNNFYPREAKVQWKVDNALQSGNSQESVTEQDSKDSTYSLSSTLTLSKADYEKHKVYACEVTHQGLSSPVTKSFNRGEC

SEQ ID NO: 39 - protein, 327 aa, artificial
  HC constant domain
ASTKGPSVFPLAPCSRSTSESTAALGCLVKDYFPEPVTVSWNSGALTSGVHTFPAVLQSSGLYSLSSVVTVPSSSLGTKTYTCNVDHKPSNTKVDKRVESKYGPPCPPCPAPEFLGGPSVFLFPPKPKDTLMISRTPEVTCVVVDVSQEDPEVQFNWYVDGVEVHNAKTKPREEQFNSTYRVVSVLTVLHQDWLNGKEYKCKVSNKGLPSSIEKTISKAKGQPREPQVYTLPPSQEEMTKNQVSLTCLVKGFYPSDIAVEWESNGQPENNYKTTPPVLDSDGSFFLYSRLTVDKSRWQEGNVFSCSVMHEALHNHYTQKSLSLSPGK

SEQ ID NO: 40 - protein, 107 aa, artificial [sequence omitted]

SEQ ID NO: 41 - protein, 30 aa, artificial
  HFR1
QIQLVQSGSELKKPGASVKVSCKASGYTFT

SEQ ID NO: 42 - protein, 14 aa, artificial
  HFR2
WVRQAPGQGLEWMG

SEQ ID NO: 43 - protein, 32 aa, artificial
  HFR3
RFVFSLDTSVSTAYLQISSLKAEDTAVYYCAR

SEQ ID NO: 44 - protein, 11 aa, artificial
  HFR4
WGQGTLVTVSS

SEQ ID NO: 45 - protein, 23 aa, artificial
  LFR1
DVVMTQSPLSLPVTLGQPASISC

SEQ ID NO: 46 - protein, 15 aa, artificial
  LFR2
WYQQRPGQSPRLLIY

SEQ ID NO: 47 - protein, 32 aa, artificial
  LFR3
GVPDRFSGSGSGTDFTLKISRVEAEDVGVYYC

SEQ ID NO: 48 - protein, 10 aa, artificial
  LFR4
FGQGTKLEIK

SEQ ID NO: 49 - protein, 19 aa, artificial
  signal peptide
MDWLWNLLFLMAAAQSIQA

SEQ ID NO: 50 - protein, 19 aa, artificial
  signal peptide
MKLPVRLLVLMFWIPASSS

SEQ ID NO: 51 - protein, 133 aa, artificial
  ECD OX40L
QVSHRYPRIQSIKVQFTEYKKEKGFILTSQKEDEIMKVQNNSVIINCDGFYLISLKGYFSQEVNISLHYQKDEEPLFQLKKVRSVNSLMVASLTYKDKVYLNVTTDNTSLDDFHVNGGELILIHQNPGEFCVL

SEQ ID NO: 52 - protein, 238 aa, artificial [sequence omitted]

SEQ ID NO: 53 - protein, 222 aa, artificial
  ECD CD86
APLKIQAYFNETADLPCQFANSQNQSLSELVVFWQDQENLVLNEVYLGKEKFDSVHSKYMGRTSFDSDSWTLRLHNLQIKDKGLYQCIIHHKKPTGMIRIHQMNSELSVLANFSQPEIVPISNITENVYINLTCSSIHGYPEPKKMSVLLRTKNSTIEYDGVMQKSQDNVTELYDVSISLSVSFPDVTSNMTIFCILETDKTRLLSSPFSIELEDPQPPPDH

SEQ ID NO: 54 - protein, 208 aa, artificial [sequence omitted]

SEQ ID NO: 55 - protein, 184 aa, artificial
  ECD 4-1BBL
REGPELSPDDPAGLLDLRQGMFAQLVAQNVLLIDGPLSWYSDPGLAGVSLTGGLSYKEDTKELVVAKAGVYYVFFQLELRRVVAGEGSGSVSLALHLQPLRSAAGAAALALTVDLPPASSEARNSAFGFQGRLLHLSAGQRLGVHLHTEARARHAWQLTQGATVLGLFRVTPEIPAGLPSPRSE

SEQ ID NO: 56 - protein, 152 aa, artificial
  ECD of IL-7
DCDIEGKDGKQYESVLMVSIDQLLDSMKEIGSNCLNNEFNFFKRHICDANKEGMFLFRAARKLRQFLKMNSTGDFDLHLLKVSEGTTILLNCTGQVKGRKPAALGEAQPTKSLEENKSLKEQKKLNDLCFLKRLLQEIKTCWNKILMGTKEH

SEQ ID NO: 57 - protein, 330 aa, artificial
  Heavy chain constant domain (IgG1m-N298A)
ASTKGPSVFPLAPSSKSTSGGTAALGCLVKDYFPEPVTVSWNSGALTSGVHTFPAVLQSSGLYSLSSVVTVPSSSLGTQTYICNVNHKPSNTKVDKKVEPKSCDKTHTCPPCPAPELLGGPSVFLFPPKPKDTLMISRTPEVTCVVVDVSHEDPEVKFNWYVDGVEVHNAKTKPREEQYASTYRVVSVLTVLHQDWLNGKEYKCKVSNKALPAPIEKTISKAKGQPREPQVYTLPPSRDELTKNQVSLTCLVKGFYPSDIAVEWESNGQPENNYKTTPPVLDSDGSFFLYSKLTVDKSRWQQGNVFSCSVMHEALHNHYTQKSLSLSPGK

SEQ ID NO: 58 - protein, 133 aa, artificial [sequence omitted]

SEQ ID NO: 59 - protein, 444 aa, artificial
  HC anti-PD1 chimeric
QIQLVQSGPELKKPGETVKISCKASGYTFTHYGMNWVKQAPGKGLKWMGWINTNTGEPTYAEEFKGRFAFSLETSASAAFLQINNLKNEDTATYFCAKEREPGMDSWGQGTSVTVSSASTKGPSVFPLAPCSRSTSESTAALGCLVKDYFPEPVTVSWNSGALTSGVHTFPAVLQSSGLYSLSSVVTVPSSSLGTKTYTCNVDHKPSNTKVDKRVESKYGPPCPPCPAPEFLGGPSVFLFPPKPKDTLMISRTPEVTCVVVDVSQEDPEVQFNWYVDGVEVHNAKTKPREEQFNSTYRVVSVLTVLHQDWLNGKEYKCKVSNKGLPSSIEKTISKAKGQPREPQVYTLPPSQEEMTKNQVSLTCLVKGFYPSDIAVEWESNGQPENNYKTTPPVLDSDGSFFLYSRLTVDKSRWQEGNVFSCSVMHEALHNHYTQKSLSLSPGK

SEQ ID NO: 60 - protein, 219 aa, artificial
  LC anti-PD1 chimeric
DVLLTQTPLSLPVSLGDQASISCRSSQNIVHANGNTYLEWYLQKPGQSPKLLIYKVSNRFSGVPDRFSGSGSGTDFTLKITRVEAEDLGVYYCFQGSHVPNTFGGGTKLEIKRTVAAPSVFIFPPSDEQLKSGTASVVCLLNNFYPREAKVQWKVDNALQSGNSQESVTEQDSKDSTYSLSSTLTLSKADYEKHKVYACEVTHQGLSSPVTKSFNRGEC

SEQ ID NO: 61 - DNA, 2670 bp, artificial
  VH VK
cagatccagctggtgcagagcggctctgagctgaagaagccaggcgcttctgtgaaggtgtcctgcaaggccagcggctacaccttcacacactatgctatgaattgggtgagacaggctccaggacagggactggagtggatgggctggatcaacaccaatacaggcgagcctacctacgctcagggctttacaggccgcttcgtgttttctctggatacctccgtgagcacagcctatctgcagatctccagcctgaaggctgaggacaccgccgtgtactattgtgctagggagagggagccaggaatggataactggggacagggcaccctggtgacagtgtcttccgctagcaccaagggcccatcggtcttccccctggcgccctgctccaggagcacctccgagagcacagccgccctgggctgcctggtcaaggactacttccccgaaccggtgacggtgtcgtggaactcaggcgccctgaccagcggcgtgcacaccttcccggctgtcctacagtcctcaggactctactccctcagcagcgtggtgaccgtgccctccagcagcttgggcacgaagacctacacctgcaacgtagatcacaagcccagcaacaccaaggtggacaagagagttgagtccaaatatggtcccccatgcccaccatgcccagcacctgagttcctggggggaccatcagtcttcctgttccccccaaaacccaaggacactctcatgatctcccggacccctgaggtcacgtgcgtggtggtggacgtgagccaggaagaccccgaggtccagttcaactggtacgtggatggcgtggaggtgcataatgccaagacaaagccgcgggaggagcagttcaacagcacgtaccgtgtggtcagcgtcctcaccgtcctgcaccaggactggctgaacggcaaggagtacaagtgcaaggtctccaacaaaggcctcccgtcctccatcgagaaaaccatctccaaagccaaagggcagccccgagagccacaggtgtacaccctgcccccatcccaggaggagatgaccaagaaccaggtcagcctgacctgcctggtcaaaggcttctaccccagcgacatcgccgtggagtgggagagcaatgggcagccggagaacaactacaagaccacgcctcccgtgctggactccgacggctccttcttcctctacagcaggctaaccgtggacaagagcaggtggcaggaggggaatgtcttctcatgctccgtgatgcatgaggctctgcacaaccactacacacagaagagcctctccctgtctccgggtaaatgacagatccagctggtgcagagcggctctgagctgaagaagccaggcgcttctgtgaaggtgtcctgcaaggccagcggctacaccttcacacactatgctatgaattgggtgagacaggctccaggacagggactggagtggatgggctggatcaacaccaatacaggcgagcctacctacgctcagggctttacaggccgcttcgtgttttctctggatacctccgtgagcacagcctatctgcagatctccagcctgaaggctgaggacaccgccgtgtactattgtgctagggagagggagccaggaatggataactggggacagggcaccctggtgacagtgtcttccgctagcaccaagggcccatcggtcttccccctggcgccctgctccaggagcacctccgagagcacagccgccctgggctgcctggtcaaggactacttccccgaaccggtgacggtgtcgtggaactcaggcgccctgaccagcggcgtgcacaccttcccggctgtcctacagtcctcaggactctactccctcagcagcgtggtgaccgtgccctccagcagcttgggcacgaagacctacacctgcaacgtagatcacaagcccagcaacaccaaggtggacaagagagttgagtccaaatatggtcccccatgcccaccatgcccagcacctgagttcctggggggaccatcagtcttcctgttccccccaaaacccaaggacactctcatgatctcccggacccctgaggtcacgtgcgtggtggtggacgtgagccaggaagaccccgaggtccagttcaactggtacgtggatggcgtggaggtgcataatgccaagacaaagccgcgggaggagcagttcaacagcacgtaccgtgtggtcagcgtcctcaccgtcctgcaccaggactggctgaacggcaaggagtacaagtgcaaggtctccaacaaaggcctcccgtcctccatcgagaaaaccatctccaaagccaaagggcagccccgagagccacaggtgtacaccctgcccccatcccaggaggagatgaccaagaaccaggtcagcctgacctgcctggtcaaaggcttctaccccagcgacatcgccgtggagtgggagagcaatgggcagccggagaacaactacaagaccacgcctcccgtgctggactccgacggctccttcttcctctacagcaggctaaccgtggacaagagcaggtggcaggaggggaatgtcttctcatgctccgtgatgcatgaggctctgcacaaccactacacacagaagagcctctccctgtctccgggtaaatga

SEQ ID NO: 62 - DNA, 660 bp, artificial
  VL-VD
gacgtggtcatgacacagagcccactgtctctgcctgtgaccctgggacagccagcctctatctcctgcagatccagccagtctctggtgcacgctaacaccaatacatacctggagtggtatcagcagaggccaggacagtccccaaggctgctgatctacaaggtgtccaacagattcagcggagtgccagaccgctttagcggatctggatccggaaccgacttcaccctgaagatctccagggtggaggctgaggatgtgggcgtgtactattgtttccagggcacccatgtgcctaatacatttggccagggcaccaagctggagatcaagcgtacggtggctgcaccatctgtcttcatcttcccgccatctgatgagcagttgaaatctggaactgcctctgttgtgtgcctgctgaataacttctatcccagagaggccaaagtacagtggaaggtggataacgccctccaatcgggtaactcccaggagagtgtcacagagcaggacagcaaggacagcacctacagcctcagcagcaccctgacgctgagcaaagcagactacgagaaacacaaagtctacgcctgcgaagtcacccatcagggcctgagctcgcccgtcacaaagagcttcaacaggggagagtgttag